European Patent Specification EP 3 813 852 B1, published July 30, 2025. Title: Methods to Induce Terminal Differentiation in Stem Cells by Interfering with DNA Replication. Methods of Inducing Pancreatic Differentiation, and Differentiated Cells Obtained Thereof. Applicant: The Trustees of Columbia University in the City of New York. Application Filed Herewith. The sequence listing filed with the application follows.

SEQUENCE LISTING (18 sequences)

SEQ ID NO: 1 - DNA, 19 bp, Artificial Sequence
  Synthetic Primer
tgggctcgagaaggatgtg

SEQ ID NO: 2 - DNA, 20 bp, Artificial Sequence
  Synthetic Primer
gcatagtcgctgcttgatcg

SEQ ID NO: 3 - DNA, 18 bp, Artificial Sequence
  Synthetic Primer
ggcgcagcagaatccaga

SEQ ID NO: 4 - DNA, 18 bp, Artificial Sequence
  Synthetic Primer
ccacgacttgcccagcat

SEQ ID NO: 5 - DNA, 18 bp, Artificial Sequence
  Synthetic Primer
gggagcggtgaagatgga

SEQ ID NO: 6 - DNA, 22 bp, Artificial Sequence
  Synthetic Primer
tcatgttgctcacggaggagta

SEQ ID NO: 7 - DNA, 20 bp, Artificial Sequence
  Synthetic Primer
ccctgggtgaccactaaacc

SEQ ID NO: 8 - DNA, 20 bp, Artificial Sequence
  Synthetic Primer
cacagcctctacctcggaac

SEQ ID NO: 9 - DNA, 20 bp, Artificial Sequence
  Synthetic Primer
attcgttggggatgacagag

SEQ ID NO: 10 - DNA, 20 bp, Artificial Sequence
  Synthetic Primer
cgagtcctgcttcttcttgg

SEQ ID NO: 11 - DNA, 21 bp, Artificial Sequence
  Synthetic Primer
tcttttctcctttggggctgg

SEQ ID NO: 12 - DNA, 20 bp, Artificial Sequence
  Synthetic Primer
tctcacgggtcacttggaca

SEQ ID NO: 13 - DNA, 20 bp, Artificial Sequence
  Synthetic Primer
gttccagcagaagcttctcg

SEQ ID NO: 14 - DNA, 20 bp, Artificial Sequence
  Synthetic Primer
gctgaaattctccccgcctt

SEQ ID NO: 15 - DNA, 20 bp, Artificial Sequence
  Synthetic Primer
ttctacacacccaagacccg

SEQ ID NO: 16 - DNA, 17 bp, Artificial Sequence
  Synthetic Primer
caatgccacgcttctgc

SEQ ID NO: 17 - DNA, 20 bp, Artificial Sequence
  Synthetic Primer
aagttcccaaagagggcttg

SEQ ID NO: 18 - DNA, 20 bp, Artificial Sequence
  Synthetic Primer
agctgccttgtaccagcatt